European Patent Specification EP 4 200 412 B1, published February 18, 2026. Title: ENGINEERED MEGANUCLEASES HAVING SPECIFICITY FOR A RECOGNITION SEQUENCE IN THE TRANSTHYRETIN GENE. Applicant: PRECISION BIOSCIENCES, INC. Application Not Yet Assigned. The sequence listing filed with the application follows.

SEQUENCE LISTING (70 sequences)

SEQ ID NO: 1 - protein, 163 aa, Chlamydomonas reinhardtii
MNTKYNKEFLLYLAGFVDGDGSIIAQIKPNQSYKFKHQLSLAFQVTQKTQRRWFLDKLVDEIGVGYVRDRGSVSDYILSEIKPLHNFLTQLQPFLKLKQKQANLVLKIIWRLPSAKESPDKFLEVCTWVDQIAALNDSKTRKTTSETVRAVLDSLSEKKKSSP

SEQ ID NO: 2 - protein, 9 aa, Chlamydomonas reinhardtii
LAGLIDADG

SEQ ID NO: 3 - DNA, 7258 bp, Homo sapiens
gttgactaagtcaataatcagaatcagcaggtttgcagtcagattggcagggataagcagcctagctcaggagaagtgagtataaaagccccaggctgggagcagccatcacagaagtccactcattcttggcaggatggcttctcatcgtctgctcctcctctgccttgctggactggtatttgtgtctgaggctggccctacggtgagtgtttctgtgacatcccattcctacatttaagattcacgctaaatgaagtagaagtgactccttccagctttgccaaccagcttttattactagggcaagggtacccagcatctatttttaatataattaattcaaacttcaaaaagaatgaagttccactgagcttactgagctgggacttgaactctgagcattctacctcattgctttggtgcattaggtttgtaatatctggtacctctgtttcctcagatagatgatagaaataaagatatgatattaaggaagctgttaatactgaattttcagaaaagtatccctccataaaatgtatttgggggacaaactgcaggagattatattctggccctatagttattcaaaacgtatttattgattaatctttaaaaggcttagtgaacaatattctagtcagatatctaattcttaaatcctctagaagaattaactaatactataaaatgggtctggatgtagttctgacattattttataacaactggtaagagggagtgactatagcaacaactaaaatgatctcaggaaaacctgtttggccctatgtatggtacattacatcttttcagtaattccactcaaatggagacttttaacaaagcaactgttctcaggggacctattttctcccttaaaattcattatacacatccctggttgatagcagtgtgtctggaggcagaaaccattcttgctttggaaacaattacgtctgtgttatactgagtagggaagctcattaattgtcgacacttacgttcctgataatgggatcagtgtgtaattcttgtttcgctccagatttctaataccacaaagaataaatcctttcactctgatcaattttgttaacttctcacgtgtcttctctacacccagggcaccggtgaatccaagtgtcctctgatggtcaaagttctagatgctgtccgaggcagtcctgccatcaatgtggccgtgcatgtgttcagaaaggctgctgatgacacctgggagccatttgcctctgggtaagttgccaaagaaccctcccacaggacttggttttatcttcccgtttgcccctcacttggtagagagaggctcacatcatctgctaaagaatttacaagtagattgaaaaacgtaggcagaggtcaagtatgccctctgaaggatgccctctttttgttttgcttagctaggaagtgaccaggaacctgagcatcatttaggggcagacagtagagaaaagaaggaatcagaactcctctcctctagctgtggtttgcaacccttttgggtcacagaacactttatgtaggtgatgaaaagtaaacattctatgcccagaaaaaatgcacagatacacacacatacaaaatcatatatgtgattttaggagtttcacagattccctggtgtccctgggtaacaccaaagctaagtgtccttgtcttagaattttaggaaaaggtataatgtgtattaacccattaacaaaaggaaaggaattcagaaatattattaaccaggcatctgtctgtagttaatatggatcacccaaaacccaaggcttttgcctaatgaacactttggggcacctactgtgtgcaaggctgggggctgtcaagctcagttaaaaaaaaaaagatagaagagatggatccatgaggcaaagtacagccccaggctaatcccacgatcacccgacttcatgtccaagagtggcttctcaccttcattagccagttcacaattttcatggagtttttctacctgcactagcaaaaacttcaaggaaaatacatattaataaatctaagcaaagtgaccagaagacagagcaatcaggagaccctttgcatccagcagaagaggaactgctaagtatttacatctccacagagaagaatttctgttgggttttaattgaaccccaagaaccacatgattcttcaaccattattgggaagatcattttcttaggtctggttttaactggctttttatttgggaattcatttatgtttatataaaatgccaagcataacatgaaaagtggttacaggactattctaagggagagacagaatggacaccaaaaatattccaatgttcttgtgaatcttttccttgcaccaggacaaaaaaaaaaagaagtgaaaagaagaaaggaggaggggcataatcagagtcagtaaagacaactgctatttttatctatcgtagctgttgcagtcaaatgggaagcaatttccaacattcaactatggagctggtacttacatggaaatagaagttgcctagtgtttgttgctggcaaagagttatcagagaggttaaatatataaaagggaaaagagtcagatacaggttcttcttcctactttaggttttccactgtgtgtgcaaatgatactccctggtggtgtgcagatgcctcaaagctatcctcacaccacaagggagaggagcgagatcctgctgtcctggagaagtgcagagttagaacagctgtggccacttgcatccaatcatcaatcttgaatcacagggactctttcttaagtaaacattatacctggccgggcacggtggctcacgcctgtaatcccagcactttgggatgccaaagtgggcatatcatctgaggtcaggagttcaagaccagcctggccaacatggcaaaactccgtctttatgaaaaatacaaaaattagccaggcatggtggcaggcgcctgtaatcccagctaattgggaggctgaggctggagaatcccttgaatctaggaggcagaggttgcagtgagctgagatcgtgccattgcactccagcctgggtgacaagagtaaaactctgtctcaaaaaaaaaaaattatacctacattctcttcttatcagagaaaaaaatctacagtgagcttttcaaaaagtttttacaaactttttgccatttaatttcagttaggagttttccctacttctgacttagttgaggggaaatgttcataacatgtttataacatgtttatgtgtgttagttggtgggggtgtattactttgccatgccatttgtttcctccatgcgtaacttaatccagactttcacaccttataggaaaaccagtgagtctggagagctgcatgggctcacaactgaggaggaatttgtagaagggatatacaaagtggaaatagacaccaaatcttactggaaggcacttggcatctccccattccatgagcatgcagaggtgagtatacagaccttcgagggttgttttggttttggtttttgcttttggcattccaggaaatgcacagttttactcagtgtaccacagaaatgtcctaaggaaggtgatgaatgaccaaaggttccctttcctattatacaagaaaaaattcacaacactctgagaagcaaatttctttttgactttgatgaaaatccacttagtaacatgacttgaacttacatgaaactactcatagtctattcattccactttatatgaatattgatgtatctgctgttgaaataatagtttatgaggcagccctccagaccccacgtagagtgtatgtaacaagagatgcaccattttatttctcgaaaacccgtaacattcttcattccaaaacacatctggcttctcggaggtctggacaagtgattcttggcaacacatacctatagagacaataaaatcaaagtaataatggcaacacaatagataacatttaccaagcatacaccatgtggcagacacaattataagtgttttccatatttaacctacttaatcctcaggaataagccactgaggtcagtcctattattatccccatcttatagatgaagaaaatgaggcaccaggaagtcaaataacttgtcaaaggtcacaagactaggaaatacacaagtagaaatgtttacaattaaggcccaggctgggtttgccctcagttctgctatgcctcgcattatgccccaggaaactttttcccttgtgaaagccaagcttaaaaaaagaaaagccacatttgtaacgtgctctgttcccctgcctatggtgaggatcttcaaacagttatacatggacccagtccccctgccttctccttaatttcttaagtcatttgaaacagatggctgtcatggaaatagaatccagacatgttggtcagagttaaagatcaactaattccatcaaaaatagctcggcatgaaagggaactattctctggcttagtcatggatgagactttcaattgctataaagtggttcctttattagacaatgttaccagggaaacaacaggggtttgtttgacttctggggcccacaagtcaacaagagagccccatctaccaaggagcatgtccctgactacccctcagccagcagcaagacatggaccccagtcagggcaggagcagggtttcggcggcgcccagcacaagacattgcccctagagtctcagcccctaccctcgagtaatagatctgcctacctgagactgttgtttgcccaagagctgggtctcagcctgatgggaaccatataaaaaggttcactgacatactgcccacatgttgttctctttcattagatcttagcttccttgtctgctcttcattcttgcagtattcattcaacaaacattaaaaaaaaaaaaaagcattctatgtgtggaacactctgctagatgctgtggatttagaaatgaaaatacatcccgacccttggaatggaagggaaaggactgaagtaagacagattaagcaggaccgtcagcccagcttgaagcccagataaatacggagaacaagagagagcgagtagtgagagatgagtcccaatgcctcactttggtgacgggtgcgtggtgggcttcatgcagcttcttctgataaatgcctccttcagaactggtcaactctaccttggccagtgacccaggtggtcatagtagatttaccaagggaaaatggaaacttttattaggagctcttaggcctcttcacttcatggatttttttttcctttttttttgagatggagttttgccctgtcacccaggctggaatgcagtggtgcaatctcagctcactgcaacctccgcctcccaggttcaagcaattctcctgcctcagcctcccgagtagctgggactacaggtgtgcgccaccacaccaggctaatttttgtattttttgtaaagacaggttttcaccacgttggccaggctggtctgaactccagacctcaggtgattcacctgtctcagcctcccaaagtgctgggattacaggtgtgagccaccgtgcccggctacttcatggatttttgattacagattatgcctcttacaatttttaagaagaatcaagtgggctgaaggtcaatgtcaccataagacaaaagacatttttattagttgattctagggaattggccttaaggggagccctttcttcctaagagattcttaggtgattctcacttcctcttgccccagtattatttttgtttttggtatggctcactcagatccttttttcctcctatccctaagtaatccgggtttctttttcccatatttagaacaaaatgtatttatgcagagtgtgtccaaacctcaacccaaggcctgtatacaaaataaatcaaattaaacacatctttactgtcttctacctctttcctgacctcaatatatcccaacttgcctcactctgagaaccaaggctgtcccagcacctgagtcgcagatattctactgatttgacagaactgtgtgactatctggaacagcattttgatccacaatttgcccagttacaaagcttaaatgagctctagtgcatgcatatatatttcaaaattccaccatgatcttccacactctgtattgtaaatagagccctgtaatgcttttacttcgtatttcattgcttgttatacataaaaatatacttttcttcttcatgttagaaaatgcaaagaataggagggtgggggaatctctgggcttggagacaggagacttgccttcctactatggttccatcagaatgtagactgggacaatacaataattcaagtctggtttgctcatctgtaaattgggaagaatgtttccagctccagaatgctaaatctctaagtctgtggttggcagccactattgcagcagctcttcaatgactcaatgcagttttgcattctccctaccttttttttctaaaaccaataaaatagatacagcctttaggctttctgggatttcccttagtcaagctagggtcatcctgactttcggcgtgaatttgcaaaacaagacctgactctgtactcctgctctaaggactgtgcatggttccaaaggcttagcttgccagcatatttgagctttttccttctgttcaaactgttccaaaatataaaagaataaaattaattaagttggcactggacttccggtggtcagtcatgtgtgtcatctgtcacgtttttcgggctctggtggaaatggatctgtctgtcttctctcataggtggtattcacagccaacgactccggcccccgccgctacaccattgccgccctgctgagcccctactcctattccaccacggctgtcgtcaccaatcccaaggaatgagggacttctcctccagtggacctgaaggacgagggatgggatttcatgtaaccaagagtattccatttttactaaagcagtgttttcacctcatatgctatgttagaagtccaggcagagacaataaaacattcctgtgaaaggcacttttcattccactttaacttgattttttaaattcccttattgtcccttccaaaaaaaagagaatcaaaattttacaaagaatcaaaggaattctagaaagtatctgggcagaacgctaggagagatccaaatttccattgtcttgcaagcaaagcacgtattaaatatgatctgcagccattaaaaagacacattctgtaaa

SEQ ID NO: 4 - protein, 147 aa, Homo sapiens
MASHRLLLLCLAGLVFVSEAGPTGTGESKCPLMVKVLDAVRGSPAINVAVHVFRKAADDTWEPFASGKTSESGELHGLTTEEEFVEGIYKVEIDTKSYWKALGISPFHEHAEVVFTANDSGPRRYTIAALLSPYSYSTTAVVTNPKE

SEQ ID NO: 5 - protein, 127 aa, Homo sapiens
GPTGTGESKCPLMVKVLDAVRGSPAINVAVHVFRKAADDTWEPFASGKTSESGELHGLTTEEEFVEGIYKVEIDTKSYWKALGISPFHEHAEVVFTANDSGPRRYTIAALLSPYSYSTTAVVTNPKE

SEQ ID NO: 6 - protein, 127 aa, Homo sapiens
GPTGTGESKCPLMVKVLDAVRGSPAINVAMHVFRKAADDTWEPFASGKTSESGELHGLTTEEEFVEGIYKVEIDTKSYWKALGISPFHEHAEVVFTANDSGPRRYTIAALLSPYSYSTTAVVTNPKE

SEQ ID NO: 7 - DNA, 22 bp, Homo sapiens
tgcatgggctcacaactgagga

SEQ ID NO: 8 - DNA, 22 bp, Homo sapiens
acgtacccgagtgttgactcct

SEQ ID NO: 9 - DNA, 22 bp, Homo sapiens
gctggactggtatttgtgtctg

SEQ ID NO: 10 - DNA, 22 bp, Homo sapiens
cgacctgaccataaacacagac

SEQ ID NO: 11 - protein, 354 aa, Artificial Sequence
  Synthesized
MNTKYNKEFLLYLAGFVDADGSIYACITPRQTHKFKHVLALGFSVIQRTRRRWFLDKLVDEIGVGYVRDRDTTSEYRLSQIKPLHNFLTQLQPFLKLKQKQANLVLKIIEQLPSAKESPDKFLEVCTWVDQIAALNDSRTRKTTSETVRAVLDSLPGSVGGLSPSQASSAASSASSSPGSGISEALRAGAGSGTGYNKEFLLYLAGFVDGDGSIYASIDPDQRSKFKHGLRLNFQVSQKTQRRWFLDKLVDEIGVGYVQDKGSVSHYILSQIKPLHNFLTQLQPFLKLKQKQANLVLKIIEQLPSAKESPDKFLEVCTWVDQIAALNDSKTRKTTSETVRAVLDSLSEKKKSSP

SEQ ID NO: 12 - protein, 354 aa, Artificial Sequence
  Synthesized
MNTKYNKEFLLYLAGFVDADGSIYACITPRQDYKFKHNLALGFSVIQRTRRRWFLDKLVDEIGVGYVRDRDTTSEYRLSQIKPLHNFLTQLQPFLKLKQKQANLVLKIIEQLPSAKESPDKFLEVCTWVDQIAALNDSRTRKTTSETVRAVLDSLPGSVGGLSPSQASSAASSASSSPGSGISEALRAGAGSGTGYNKEFLLYLAGFVDGDGSIYASIDPDQRSKFKHGLRLNFQVSQKTQRRWFLDKLVDEIGVGYVQDKGSVSHYILSEIKPLHNFLTQLQPFLKLKQKQANLVLKIIEQLPSAKESPDKFLEVCTWVDQIAALNDSKTRKTTSETVRAVLDSLSEKKKSSP

SEQ ID NO: 13 - protein, 354 aa, Artificial Sequence
  Synthesized
MNTKYNKEFLLYLAGFVDADGSIYACITPRQLCKFKHGLALGFSVIQRTRRRWFLDKLVDEIGVGYVRDRDTTSEYRLSQIKPLHNFLTQLQPFLKLKQKQANLVLKIIEQLPSAKESPDKFLEVCTWVDQIAALNDSRTRKTTSETVRAVLDSLPGSVGGLSPSQASSAASSASSSPGSGISEALRAGAGSGTGYNKEFLLYLAGFVDGDGSIYASIDPDQRSKFKHGLRLNFQVSQKTQRRWFLDKLVDEIGVGYVQDKGSVSHYILSEIKPLHNFLTQLQPFLKLKQKQANLVLKIIEQLPSAKESPDKFLEVCTWVDQIAALNDSKTRKTTSETVRAVLDSLSEKKKSSP

SEQ ID NO: 14 - protein, 354 aa, Artificial Sequence
  Synthesized
MNTKYNKEFLLYLAGFVDADGSIYACITPRQTHKFKHNLALGFSVIQRTRRRWFLDKLVDEIGVGYVRDRDTTSEYRLSQIKPLHNFLTQLQPFLKLKQKQANLVLKIIEQLPSAKESPDKFLEVCTWVDQIAALNDSRTRKTTSETVRAVLDSLPGSVGGLSPSQASSAASSASSSPGSGISEALRAGAGSGTGYNKEFLLYLAGFVDGDGSIYASIDPDQRSKFKHGLRLNFQVSQKTQRRWFLDKLVDEIGVGYVQDKGSVSHYILSEIKPLHNFLTQLQPFLKLKQKQANLVLKIIEQLPSAKESPDKFLEVCTWVDQIAALNDSKTRKTTSETVRAVLDSLSEKKKSSP

SEQ ID NO: 15 - protein, 354 aa, Artificial Sequence
  Synthesized
MNTKYNKEFLLYLAGFVDGDGSIFASIEPAQRAKFKHYLRLVFNVTQKTQRRWFLDKLVDEIGVGYVSDSGSVSLYKLSEIKPLHNFLTQLQPFLKLKQKQANLVLKIIEQLPSAKESPDKFLEVCTWVDQIAALNDSKTRKTTSETVRAVLDSLPGSVGGLSPSQASSAASSASSSPGSGISEALRAGAGSGTGYNKEFLLYLAGFVDSDGSIFASIVPDQSRKFKHALRLRFIVSQNTRRRWFLDKLVDEIGVGYVKDSGRSAHYTLSEIKPLHNFLTQLQPFLKLKQKQANLVLKIIEQLPSAKESPDKFLEVCTWVDQIAALNDSKTRKTTSETVRAVLDSLSEKKKSSP

SEQ ID NO: 16 - protein, 147 aa, Artificial Sequence
  Synthesized
KEFLLYLAGFVDADGSIYACITPRQTHKFKHVLALGFSVIQRTRRRWFLDKLVDEIGVGYVRDRDTTSEYRLSQIKPLHNFLTQLQPFLKLKQKQANLVLKIIEQLPSAKESPDKFLEVCTWVDQIAALNDSRTRKTTSETVRAVLD

SEQ ID NO: 17 - protein, 147 aa, Artificial Sequence
  Synthesized
KEFLLYLAGFVDADGSIYACITPRQDYKFKHNLALGFSVIQRTRRRWFLDKLVDEIGVGYVRDRDTTSEYRLSQIKPLHNFLTQLQPFLKLKQKQANLVLKIIEQLPSAKESPDKFLEVCTWVDQIAALNDSRTRKTTSETVRAVLD

SEQ ID NO: 18 - protein, 147 aa, Artificial Sequence
  Synthesized
KEFLLYLAGFVDADGSIYACITPRQLCKFKHGLALGFSVIQRTRRRWFLDKLVDEIGVGYVRDRDTTSEYRLSQIKPLHNFLTQLQPFLKLKQKQANLVLKIIEQLPSAKESPDKFLEVCTWVDQIAALNDSRTRKTTSETVRAVLD

SEQ ID NO: 19 - protein, 147 aa, Artificial Sequence
  Synthesized
KEFLLYLAGFVDADGSIYACITPRQTHKFKHNLALGFSVIQRTRRRWFLDKLVDEIGVGYVRDRDTTSEYRLSQIKPLHNFLTQLQPFLKLKQKQANLVLKIIEQLPSAKESPDKFLEVCTWVDQIAALNDSRTRKTTSETVRAVLD

SEQ ID NO: 20 - protein, 147 aa, Artificial Sequence
  Synthesized
KEFLLYLAGFVDGDGSIYASIDPDQRSKFKHGLRLNFQVSQKTQRRWFLDKLVDEIGVGYVQDKGSVSHYILSQIKPLHNFLTQLQPFLKLKQKQANLVLKIIEQLPSAKESPDKFLEVCTWVDQIAALNDSKTRKTTSETVRAVLD

SEQ ID NO: 21 - protein, 147 aa, Artificial Sequence
  Synthesized
KEFLLYLAGFVDGDGSIYASIDPDQRSKFKHGLRLNFQVSQKTQRRWFLDKLVDEIGVGYVQDKGSVSHYILSEIKPLHNFLTQLQPFLKLKQKQANLVLKIIEQLPSAKESPDKFLEVCTWVDQIAALNDSKTRKTTSETVRAVLD

SEQ ID NO: 22 - protein, 147 aa, Artificial Sequence; identical to SEQ ID NO: 21
  Synthesized

SEQ ID NO: 23 - protein, 147 aa, Artificial Sequence; identical to SEQ ID NO: 21
  Synthesized

SEQ ID NO: 24 - protein, 147 aa, Artificial Sequence
  Synthesized
KEFLLYLAGFVDGDGSIFASIEPAQRAKFKHYLRLVFNVTQKTQRRWFLDKLVDEIGVGYVSDSGSVSLYKLSEIKPLHNFLTQLQPFLKLKQKQANLVLKIIEQLPSAKESPDKFLEVCTWVDQIAALNDSKTRKTTSETVRAVLD

SEQ ID NO: 25 - protein, 147 aa, Artificial Sequence
  Synthesized
KEFLLYLAGFVDSDGSIFASIVPDQSRKFKHALRLRFIVSQNTRRRWFLDKLVDEIGVGYVKDSGRSAHYTLSEIKPLHNFLTQLQPFLKLKQKQANLVLKIIEQLPSAKESPDKFLEVCTWVDQIAALNDSKTRKTTSETVRAVLD

SEQ ID NO: 26 - DNA, 9 bp, Homo sapiens
tgcatgggc

SEQ ID NO: 27 - DNA, 9 bp, Homo sapiens
acgtacccg

SEQ ID NO: 28 - DNA, 9 bp, Homo sapiens
aactgagga

SEQ ID NO: 29 - DNA, 9 bp, Homo sapiens
ttgactcct

SEQ ID NO: 30 - DNA, 9 bp, Homo sapiens
gctggactg

SEQ ID NO: 31 - DNA, 9 bp, Homo sapiens
cgacctgac

SEQ ID NO: 32 - DNA, 9 bp, Homo sapiens
ttgtgtctg

SEQ ID NO: 33 - DNA, 9 bp, Homo sapiens
aacacagac

SEQ ID NO: 34 - DNA, 24 bp, Artificial Sequence
  Synthesized
cactggactggtatttgtgtctga

SEQ ID NO: 35 - DNA, 24 bp, Artificial Sequence
  Synthesized
tgctggactggtatttgtgtctga

SEQ ID NO: 36 - DNA, 20 bp, Artificial Sequence
  Synthesized
ccactcattcttggcaggat

SEQ ID NO: 37 - DNA, 21 bp, Artificial Sequence
  Synthesized
cacagaaacactcaccgtagg

SEQ ID NO: 38 - DNA, 24 bp, Artificial Sequence
  Synthesized
aaattcctcctcagttgtgagccc

SEQ ID NO: 39 - DNA, 17 bp, Artificial Sequence
  Synthesized
agtctggagagctgcat

SEQ ID NO: 40 - DNA, 24 bp, Artificial Sequence
  Synthesized
ccagtaagatttggtgtctatttc

SEQ ID NO: 41 - DNA, 24 bp, Artificial Sequence
  Synthesized
atgggctcacaactgaggaggaat

SEQ ID NO: 42 - DNA, 22 bp, Artificial Sequence
  Synthesized
tccagactttcacaccttatag

SEQ ID NO: 43 - DNA, 23 bp, Artificial Sequence
  Synthesized
tccactttgtatatcccttctac

SEQ ID NO: 44 - DNA, 24 bp, Artificial Sequence
  Synthesized
tgctggactggtatttgtgtctga

SEQ ID NO: 45 - DNA, 20 bp, Artificial Sequence
  Synthesized
ccactcattcttggcaggat

SEQ ID NO: 46 - DNA, 21 bp, Artificial Sequence
  Synthesized
cacagaaacactcaccgtagg

SEQ ID NO: 47 - DNA, 19 bp, Artificial Sequence
  Synthesized
gtgtctgtctgcacatttc

SEQ ID NO: 48 - DNA, 22 bp, Artificial Sequence
  Synthesized
agaaggcacttcttctttatct

SEQ ID NO: 49 - DNA, 25 bp, Artificial Sequence
  Synthesized
cctcgctggactggtatttgtgtct

SEQ ID NO: 50 - DNA, 28 bp, Artificial Sequence
  Synthesized
tccgatactctaatctccctaggcaagg

SEQ ID NO: 51 - DNA, 17 bp, Artificial Sequence
  Synthesized
agtctggagagctgcat

SEQ ID NO: 52 - DNA, 24 bp, Artificial Sequence
  Synthesized
ccagtaagatttggtgtctatttc

SEQ ID NO: 53 - DNA, 19 bp, Artificial Sequence
  Synthesized
cctcagttgtgagcccatg

SEQ ID NO: 54 - DNA, 20 bp, Artificial Sequence
  Synthesized
ccactcgttcttggcaggat

SEQ ID NO: 55 - DNA, 21 bp, Artificial Sequence
  Synthesized
cacagaaacactcaccgtagg

SEQ ID NO: 56 - DNA, 24 bp, Artificial Sequence
  Synthesized
tgctggactggtatttgtgtctga

SEQ ID NO: 57 - DNA, 19 bp, Artificial Sequence
  Synthesized
ggatccgtgggaggtctat

SEQ ID NO: 58 - DNA, 17 bp, Artificial Sequence
  Synthesized
acctgctccagctctga

SEQ ID NO: 59 - DNA, 22 bp, Artificial Sequence
  Synthesized
tgcttcggagatccctgaaccc

SEQ ID NO: 60 - DNA, 16 bp, Artificial Sequence
  Synthesized
accgccaaggatgcac

SEQ ID NO: 61 - DNA, 16 bp, Artificial Sequence
  Synthesized
gcgggtgggaatggag

SEQ ID NO: 62 - DNA, 19 bp, Artificial Sequence
  Synthesized
ccagcaggccaggtacacc

SEQ ID NO: 63 - DNA, 24 bp, Artificial Sequence
  Synthesized
gccatgccatttgtttcctccatg

SEQ ID NO: 64 - DNA, 18 bp, Artificial Sequence
  Synthesized
gcatgctcatggaatggg

SEQ ID NO: 65 - protein, 42 aa, Artificial Sequence
  Synthesized
SLPGSVGGLSPSQASSAASSASSSPGSGISEALRAGAGSGTG

SEQ ID NO: 66 - DNA, 1065 bp, Artificial Sequence
  Synthesized
atgaatacaaaatataataaagagttcttactctacttagcagggtttgtagacgctgacggttccatctatgcctgtatcacgcctcgtcaaactcataagttcaagcacgttctggcgctcgggttctcagtcattcagcgtacacgtcgccgttggttcctcgacaagctggtggacgagatcggtgtgggttacgtgcgtgacagggatacgaccagcgaatacagactgtcccagatcaagcctttgcataattttttaacacaactacaaccttttctaaaactaaaacaaaaacaagcaaatttagttttaaaaattattgaacaacttccgtcagcaaaagaatccccggacaaattcttagaagtttgtacatgggtggatcaaattgcagctctgaatgattcgaggacgcgtaaaacaacttctgaaaccgttcgtgctgtgctagacagtttaccaggatccgtgggaggtctatcgccatctcaggcatccagcgccgcatcctcggcttcctcaagcccgggttcagggatctccgaagcactcagagctggagcaggttccggcactggatacaacaaggaattcctgctctacctggcgggcttcgtcgacggggacggctccatctatgccagtatcgatcctgatcaacggagtaagttcaagcacgggctgaggctcaatttccaggtctctcagaagacacagcgccgttggttcctcgacaagctggtggacgagatcggtgtgggttacgtgcaggacaagggcagcgtctcccattacattctgtcccagatcaagcctctgcacaacttcctgacccagctccagcccttcctgaagctcaagcagaagcaggccaacctcgtgctgaagatcatcgagcagctgccctccgccaaggaatccccggacaagttcctggaggtgtgcacctgggtggaccagatcgccgctctgaacgactccaagacccgcaagaccacttccgaaaccgtccgcgccgttctagacagtctctccgagaagaagaagtcgtccccctaa

SEQ ID NO: 67 - DNA, 1065 bp, Artificial Sequence
  Synthesized
atgaatacaaaatataataaagagttcttactctacttagcagggtttgtagacgctgacggttccatctatgcctgtatcacgcctcgtcaagattataagttcaagcacaatctggcgctcgggttcagtgtcattcagcgtacacgtcgccgttggttccttgacaagctggtggacgagatcggtgtgggttacgtgcgtgacagggatacgaccagcgaatacagactgtcccagatcaagcctttgcataattttttaacacaactacaaccttttctaaaactaaaacaaaaacaagcaaatttagttttaaaaattattgaacaacttccgtcagcaaaagaatccccggacaaattcttagaagtttgtacatgggtggatcaaattgcagctctgaatgattcgaggacgcgtaaaacaacttctgaaaccgttcgtgctgtgctagacagtttaccaggatccgtgggaggtctatcgccatctcaggcatccagcgccgcatcctcggcttcctcaagcccgggttcagggatctccgaagcactcagagctggagcaggttccggcactggatacaacaaggaattcctgctctacctggcgggcttcgtcgacggggacggctccatctatgccagtatcgatcctgatcaacggagtaagttcaagcacgggctgaggctcaatttccaggtctctcagaagacacagcgccgttggttcctcgacaagctggtggacgagatcggtgtgggttacgtgcaggacaagggcagcgtctcccattacattctgtccgagatcaagcctctgcacaacttcctgacccagctccagcccttcctgaagctcaagcagaagcaggccaacctcgtgctgaagatcatcgagcagctgccctccgccaaggaatccccggacaagttcctggaggtgtgcacctgggtggaccagatcgccgctctgaacgactccaagacccgcaagaccacttccgaaaccgtccgcgccgttctagacagtctctccgagaagaagaagtcgtccccctaa

SEQ ID NO: 68 - DNA, 1065 bp, Artificial Sequence
  Synthesized
atgaatacaaaatataataaagagttcttactctacttagcagggtttgtagacgctgacggttccatctatgcctgtatcacgcctcgtcaactttgtaagttcaagcacgggctggcgctcgggttctcggtcattcagcgtacacgtcgccgttggttcctcgacaagctggtggacgagatcggtgtgggttacgtgcgtgacagggatacgaccagcgaatacagactgtcccagatcaagcctttgcataattttttaacacaactacaaccttttctaaaactaaaacaaaaacaagcaaatttagttttaaaaattattgaacaacttccgtcagcaaaagaatccccggacaaattcttagaagtttgtacatgggtggatcaaattgcagctctgaatgattcgaggacgcgtaaaacaacttctgaaaccgttcgtgctgtgctagacagtttaccaggatccgtgggaggtctatcgccatctcaggcatccagcgccgcatcctcggcttcctcaagcccgggttcagggatctccgaagcactcagagctggagcaggttccggcactggatacaacaaggaattcctgctctacctggcgggcttcgtcgacggggacggctccatctatgccagtatcgatcctgatcaacggagtaagttcaagcacgggctgaggctcaatttccaggtctctcagaagacacagcgccgttggttcctcgacaagctggtggacgagatcggtgtgggttacgtgcaggacaagggcagcgtctcccattacattctgtccgagatcaagcctctgcacaacttcctgacccagctccagcccttcctgaagctcaagcagaagcaggccaacctcgtgctgaagatcatcgagcagctgccctccgccaaggaatccccggacaagttcctggaggtgtgcacctgggtggaccagatcgccgctctgaacgactccaagacccgcaagaccacttccgaaaccgtccgcgccgttctagacagtctctccgagaagaagaagtcgtccccctaa

SEQ ID NO: 69 - DNA, 1065 bp, Artificial Sequence
  Synthesized
atgaatacaaaatataataaagagttcttactctacttagcagggtttgtagacgctgacggttccatctatgcctgtatcacgcctcgtcaaacgcataagttcaagcacaatctggcgctcgggttcagtgtcattcagcgtacacgtcgccgttggttccttgacaagctggtggacgagatcggtgtgggttacgtgcgtgacagggatacgaccagcgaatacagactgtcccagatcaagcctttgcataattttttaacacaactacaaccttttctaaaactaaaacaaaaacaagcaaatttagttttaaaaattattgaacaacttccgtcagcaaaagaatccccggacaaattcttagaagtttgtacatgggtggatcaaattgcagctctgaatgattcgaggacgcgtaaaacaacttctgaaaccgttcgtgctgtgctagacagtttaccaggatccgtgggaggtctatcgccatctcaggcatccagcgccgcatcctcggcttcctcaagcccgggttcagggatctccgaagcactcagagctggagcaggttccggcactggatacaacaaggaattcctgctctacctggcgggcttcgtcgacggggacggctccatctatgccagtatcgatcctgatcaacggagtaagttcaagcacgggctgaggctcaatttccaggtctctcagaagacacagcgccgttggttcctcgacaagctggtggacgagatcggtgtgggttacgtgcaggacaagggcagcgtctcccattacattctgtccgagatcaagcctctgcacaacttcctgacccagctccagcccttcctgaagctcaagcagaagcaggccaacctcgtgctgaagatcatcgagcagctgccctccgccaaggaatccccggacaagttcctggaggtgtgcacctgggtggaccagatcgccgctctgaacgactccaagacccgcaagaccacttccgaaaccgtccgcgccgttctagacagtctctccgagaagaagaagtcgtccccctaa

SEQ ID NO: 70 - DNA, 1065 bp, Artificial Sequence
  Synthesized
atgaatacaaaatataataaagagttcttactctacttagcagggtttgtagacggtgacggttccatcttcgcctccattgaaccagcgcaacgggcgaagttcaagcactatctgcgtctcgtgttcaatgtcactcagaagacacagcgccgttggttcctcgacaagctggtggacgagatcggtgtgggttacgtgtctgactctggcagcgtctccctttacaagctcagcgaaattaaaccattgcataattttttaacacaactacaaccttttctaaaactaaaacaaaaacaagcaaatttagttttaaaaattattgaacaacttccgtcagcaaaagaatccccggacaaattcttagaagtttgtacatgggtggatcaaattgcagctctgaatgattcgaagacgcgtaaaacaacttctgaaaccgttcgtgctgtgctagacagtttaccaggatccgtgggaggtctatcgccatctcaggcatccagcgccgcatcctcggcttcctcaagcccgggttcagggatctccgaagcactcagagctggagcaggttccggcactggatacaacaaggaattcctgctctacctggcgggcttcgtcgacagcgacggctccatctttgccagtatcgtgcctgatcaatcgcgtaagttcaagcatgctctccggttgcgctttattgtcagtcagaatacaaggcgccgttggttcctcgacaagctggtggacgagatcggtgtgggttacgtgaaggactctggtcggagcgcccattatactctgtccgagatcaagcctctgcacaacttcctgacccagctccagcccttcctgaagctcaagcagaagcaggccaacctcgtgctgaagatcatcgagcagctgccctccgccaaggaatccccggacaagttcctggaggtgtgcacctgggtggaccagatcgccgctctgaacgactccaagacccgcaagaccacttccgaaaccgtccgcgccgttctagacagtctctccgagaagaagaagtcgtccccctaa